European Patent Specification EP 3 470 528 B1, published September 25, 2024. Title: Method of predicting effect of medicinal therapy on cancer. Applicant: NATIONAL CANCER CENTER SRL, INC. FUJIREBIO INC. The sequence listing filed with the application follows.

SEQUENCE LISTING (2 sequences)

SEQ ID NO: 1 - DNA, 120 bp, Homo sapiens
  CpG_site (102)..(103): cg15896301 target site of HSD17B4
cgcgctctgcgctcatcttcctaccagaaatcggcaagtcactgaccctcgtcccgcccccgccattccccgcctcctcctgtcccgcagtcggcgtccagcggctctgcttgttcgtgt

SEQ ID NO: 2 - DNA, 2001 bp, Homo sapiens
  CpG_site (1092)..(1093): cg15896301 target site of HSD17B4
tttgggaactgataaatgtccgtgaaatcttcacaatttatgttcctctgctgcggctctagcaggtccctctgtttggggtccatgacttcccgcaacatccaatcaatcctccataatgggcaaagtgatctttccatagtgtaaatgtgttcccaccactctctggagtaatcctacttaaaaccgttttcagcacaaaattcaaacatctaaacatgatcttgctggctttgcttttgtggctttaccctctttctccccaaacctagctagtgtttgtgctgcctgtaatgcccttctttctttgcaggggtcgccactttaggtcctggtcctccttcagaaagtttttcctctttctccccagcggggatagggtctgtttattttgacaccattagctcacttacacacattggtcacaagtctaggctgcaccgttattgaaagtttaccatctgactctgagtagcttgaggatcctatcaaaactcaggagatgctcagtaaatgttgattgaactatgactgttctcaacatacaaacgcaagatcatttaggaacacttgtcaaaatgtttttgccccttgagattctattttgggaggtaagcagtgggggtccaggactctgcattttgacagtcccctgatgtttgcatgtagaagtgcagggattattacactgacaaatctttaccatccctaagggggactttccttcccaggggctatctctggaagcccctcaaggataggggccgcatgctgtttctctaggtcagcaactaaacccagaaaacgtttattgagtgaatgatgaaacgacaggtgaatagatgaacgcaaggtgtcgagttaactattcttctacacaagtcctagcagctcccattgcttccagccgcagaaatggcccctggaaggcaagtcttccagcgagtggagtcactcttaactacatttcccaggattccaagggagccgcgcgctctgcgctcatcttcctaccagaaatcggcaagtcactgaccctcgtcccgcccccgccattccccgcctcctcctgtcccgcagtcggcgtccagcggctctgcttgttcgtgtgtgtgtcgttgcaggccttattcatgggctcaccgctgaggttcgacgggcgggtggtactggtcaccggcgcgggggcaggtgagcatgcgaaggttggaggccgcgccccttgctgaggcgcagctggctgctcttttcgggccggcatacgcgcgcagccgcagctgaggtcaccccgctgaggtggtggggaggggaatggttattcttgaggcaccgcatctcttgaggaggaaagagccggaaacacctggtctctcaagcaggtacagcccgcttctccccagcaccccggtgtgggcttcccaaggtcctgcctgagaggagaggccaggctgggctgctgattgcaaaactgggtgaaagttctccctgacccttatctgtgggcatcgattgttactcttcctgcaattaactctcttagatctttgcctagtcttttaaaggactgaaaagccgcgaggggcgggggctggaattcgccccctgaagcgcagagatgtcagctcctgaaaagtcattcggtcgttcagtgtttgtttccctctgtcgtaagattttaagttcgtgagaggaccttctttaaagagggcgtctgataagagcccttccccgttggagtttgtatgcttagcaagtcacaatctgttctcgaaatccactggagtcttggcagaggttgtaagctcaaatgcgcacaggggtcaggcgtatgatggagaaagaaaatgggagtaggatgggcacatctgaggaactggagagcagagaattccgaagtggaccggccagtgggaaagttgcctgtatttcaggagcggcaaaatggaaaattgttatgtgaaatagccccattttttaaagtacaaaaaattaaaacaaacc